European Patent Application EP 4 389 772 A1, published June 26, 2024. Title: TARGETED DELIVERY OF THERAPEUTIC ENZYMES. Applicant: JOINT-STOCK COMPANY "GENERIUM". Application WO. The sequence listing filed with the application follows.

SEQUENCE LISTING (15 sequences)

SEQ ID NO: 1 - protein, 124 aa, synthetic construct
  source 1..124: note = Insulin receptor epitope recognized by an IgG immunoglobulin
MEEVSGTKGRQERNDIALKTNGDQASCENELLKFSYIRTSFDKILLRWEPYWPPDFRDLLGFMLFYKEAPYQNVTEFDGQDACGSNSWTVVDIDPPLRSNDPKSQNHPGWLMRGLKPWTQYAIF

SEQ ID NO: 2 - protein, 214 aa, synthetic construct
  source 1..214: note = Immunoglobulin IgG light chain to the insulin receptor
DIQMTQSPSSLSASLGERVSLTCRASQDIGGNLYWLQQGPDGTIKRLIYATSSLDSGVPKRFSGSRSGSDYSLTISSLESEDFVDYYCLQYSSSPWTFGGGTKMEIKRTVAAPSVFIFPPSDEQLKSGTASVVCLLNNFYPREAKVQWKVDNALQSGNSQESVTEQDSKDSTYSLSSTLTLSKADYEKHKVYACEVTHQGLSSPVTKSFNRGEC

SEQ ID NO: 3 - protein, 221 aa, synthetic construct
  source 1..221: note = Fragment VH-CH1 of the immunoglobulin IgG heavy chain to the insulin receptor
QVQLQQSGPELVKPGALVKISCKASGYTFTNYDIHWVKQRPGQGLEWIGWIYPGDGSTKYNEKFKGKATLTADKSSSTAYMHLSSLTSEKSAVYFCAREWAYWGQGTLVTVSAASTKGPSVFPLAPSSKSTSGGTAALGCLVKDYFPEPVTVSWNSGALTSGVHTFPAVLQSSGLYSLSSVVTVPSSSLGTQTYICNVNHKPSNTKVDKKVEPKSCDKTHL

SEQ ID NO: 4 - protein, 748 aa, synthetic construct
  source 1..748: note = Fragment VH-CH1 of the immunoglobulin IgG heavy chain to the insulin receptor coupled to an iduronate-2-sulfatase sequence
QVQLQQSGPELVKPGALVKISCKASGYTFTNYDIHWVKQRPGQGLEWIGWIYPGDGSTKYNEKFKGKATLTADKSSSTAYMHLSSLTSEKSAVYFCAREWAYWGQGTLVTVSAASTKGPSVFPLAPSSKSTSGGTAALGCLVKDYFPEPVTVSWNSGALTSGVHTFPAVLQSSGLYSLSSVVTVPSSSLGTQTYICNVNHKPSNTKVDKKVEPKSCDKTHLSSSETQANSTTDALNVLLIIVDDLRPSLGCYGDKLVRSPNIDQLASHSLLFQNAFAQQAVCAPSRVSFLTGRRPDTTRLYDFNSYWRVHAGNFSTIPQYFKENGYVTMSVGKVFHPGISSNHTDDSPYSWSFPPYHPSSEKYENTKTCRGPDGELHANLLCPVDVLDVPEGTLPDKQSTEQAIQLLEKMKTSASPFFLAVGYHKPHIPFRYPKEFQKLYPLENITLAPDPEVPDGLPPVAYNPWMDIRQREDVQALNISVPYGPIPVDFQRKIRQSYFASVSYLDTQVGRLLSALDDLQLANSTIIAFTSDHGWALGEHGEWAKYSNFDVATHVPLIFYVPGRTASLPEAGEKLFPYLDPFDSASQLMEPGRQSMDLVELVSLFPTLAGLAGLQVPPRCPVPSFHVELCREGKNLLKHFRFRDLEEDPYLPGNPRELIAYSQYPRPSDIPQWNSDKPSLKDIKIMGYSIRTIDYRYTVWVGFNPDEFLANFSDIHAGELYFVDSDPLQDHNMYNDSQGGDLFQLLMP

SEQ ID NO: 5 - protein, 760 aa, synthetic construct
  source 1..760: note = Fragment VH-CH1 of the immunoglobulin IgG heavy chain to the insulin receptor coupled to the iduronate-2-sulfatase sequence by a linker composed of glycine and serine
QVQLQQSGPELVKPGALVKISCKASGYTFTNYDIHWVKQRPGQGLEWIGWIYPGDGSTKYNEKFKGKATLTADKSSSTAYMHLSSLTSEKSAVYFCAREWAYWGQGTLVTVSAASTKGPSVFPLAPSSKSTSGGTAALGCLVKDYFPEPVTVSWNSGALTSGVHTFPAVLQSSGLYSLSSVVTVPSSSLGTQTYICNVNHKPSNTKVDKKVEPKSCDKTHGGGGSGGGGSGGGGSSETQANSTTDALNVLLIIVDDLRPSLGCYGDKLVRSPNIDQLASHSLLFQNAFAQQAVCAPSRVSFLTGRRPDTTRLYDFNSYWRVHAGNFSTIPQYFKENGYVTMSVGKVFHPGISSNHTDDSPYSWSFPPYHPSSEKYENTKTCRGPDGELHANLLCPVDVLDVPEGTLPDKQSTEQAIQLLEKMKTSASPFFLAVGYHKPHIPFRYPKEFQKLYPLENITLAPDPEVPDGLPPVAYNPWMDIRQREDVQALNISVPYGPIPVDFQRKIRQSYFASVSYLDTQVGRLLSALDDLQLANSTIIAFTSDHGWALGEHGEWAKYSNFDVATHVPLIFYVPGRTASLPEAGEKLFPYLDPFDSASQLMEPGRQSMDLVELVSLFPTLAGLAGLQVPPRCPVPSFHVELCREGKNLLKHFRFRDLEEDPYLPGNPRELIAYSQYPRPSDIPQWNSDKPSLKDIKIMGYSIRTIDYRYTVWVGFNPDEFLANFSDIHAGELYFVDSDPLQDHNMYNDSQGGDLFQLLMP

SEQ ID NO: 6 - protein, 850 aa, synthetic construct
  source 1..850: note = Fragment VH-CH1 of the immunoglobulin heavy chain to the human insulin receptor coupled to an alpha-L-iduronidase sequence
QVQLQQSGPELVKPGALVKISCKASGYTFTNYDIHWVKQRPGQGLEWIGWIYPGDGSTKYNEKFKGKATLTADKSSSTAYMHLSSLTSEKSAVYFCAREWAYWGQGTLVTVSAASTKGPSVFPLAPSSKSTSGGTAALGCLVKDYFPEPVTVSWNSGALTSGVHTFPAVLQSSGLYSLSSVVTVPSSSLGTQTYICNVNHKPSNTKVDKKVEPKSCDKTHLSSEAPHLVQVDAARALWPLRRFWRSTGFCPPLPHSQADQYVLSWDQQLNLAYVGAVPHRGIKQVRTHWLLELVTTRGSTGRGLSYNFTHLDGYLDLLRENQLLPGFELMGSASGHFTDFEDKQQVFEWKDLVSSLARRYIGRYGLAHVSKWNFETWNEPDHHDFDNVSMTMQGFLNYYDACSEGLRAASPALRLGGPGDSFHTPPRSPLSWGLLRHCHDGTNFFTGEAGVRLDYISLHRKGARSSISILEQEKVVAQQIRQLFPKFADTPIYNDEADPLVGWSLPQPWRADVTYAAMVVKVIAQHQNLLLANTTSAFPYALLSNDNAFLSYHPHPFAQRTLTARFQVNNTRPPHVQLLRKPVLTAMGLLALLDEEQLWAEVSQAGTVLDSNHTVGVLASAHRPQGPADAWRAAVLIYASDDTRAHPNRSVAVTLRLRGVPPGPGLVYVTRYLDNGLCSPDGEWRRLGRPVFPTAEQFRRMRAAEDPVAAAPRPLPAGGRLTLRPALRLPSLLLVHVCARPEKPPGQVTRLRALPLTQGQLVLVWSDEHVGSKCLWTYEIQFSQDGKAYTPVSRKPSTFNLFVFSPDTGAVSGSYRVRALDYWARPGPFSDPVPYLEVPVPRGPPSPGNP

SEQ ID NO: 7 - protein, 862 aa, synthetic construct
  source 1..862: note = Fragment VH-CH1 of the immunoglobulin heavy chain to the human insulin receptor coupled to the alpha-L-iduronidase sequence by a linker composed of glycine and serine
QVQLQQSGPELVKPGALVKISCKASGYTFTNYDIHWVKQRPGQGLEWIGWIYPGDGSTKYNEKFKGKATLTADKSSSTAYMHLSSLTSEKSAVYFCAREWAYWGQGTLVTVSAASTKGPSVFPLAPSSKSTSGGTAALGCLVKDYFPEPVTVSWNSGALTSGVHTFPAVLQSSGLYSLSSVVTVPSSSLGTQTYICNVNHKPSNTKVDKKVEPKSCDKTHGGGGSGGGGSGGGGSEAPHLVQVDAARALWPLRRFWRSTGFCPPLPHSQADQYVLSWDQQLNLAYVGAVPHRGIKQVRTHWLLELVTTRGSTGRGLSYNFTHLDGYLDLLRENQLLPGFELMGSASGHFTDFEDKQQVFEWKDLVSSLARRYIGRYGLAHVSKWNFETWNEPDHHDFDNVSMTMQGFLNYYDACSEGLRAASPALRLGGPGDSFHTPPRSPLSWGLLRHCHDGTNFFTGEAGVRLDYISLHRKGARSSISILEQEKVVAQQIRQLFPKFADTPIYNDEADPLVGWSLPQPWRADVTYAAMVVKVIAQHQNLLLANTTSAFPYALLSNDNAFLSYHPHPFAQRTLTARFQVNNTRPPHVQLLRKPVLTAMGLLALLDEEQLWAEVSQAGTVLDSNHTVGVLASAHRPQGPADAWRAAVLIYASDDTRAHPNRSVAVTLRLRGVPPGPGLVYVTRYLDNGLCSPDGEWRRLGRPVFPTAEQFRRMRAAEDPVAAAPRPLPAGGRLTLRPALRLPSLLLVHVCARPEKPPGQVTRLRALPLTQGQLVLVWSDEHVGSKCLWTYEIQFSQDGKAYTPVSRKPSTFNLFVFSPDTGAVSGSYRVRALDYWARPGPFSDPVPYLEVPVPRGPPSPGNP

SEQ ID NO: 8 - protein, 214 aa, synthetic construct
  source 1..214: note = Immunoglobulin IgG light chain to the insulin receptor LFR1
DIQMTQSPSSLSASVGDRVTITCRASQDIGGNLYWYQQKPGKAPKLLIYATSSLDSGVPSRFSGSGSGTDFTLTISSLQPEDVATYYCLQYSSSPWTFGQGTKVEIKRTVAAPSVFIFPPSDEQLKSGTASVVCLLNNFYPREAKVQWKVDNALQSGNSQESVTEQDSKDSTYSLSSTLTLSKADYEKHKVYACEVTHQGLSSPVTKSFNRGEC

SEQ ID NO: 9 - protein, 214 aa, synthetic construct
  source 1..214: note = Immunoglobulin IgG light chain to the insulin receptor LFR2
EIVLTQSPDFQSVTPKEKVTITCRASQDIGGNLYWYQQKPDQSPKLLIKATSSLDSGVPSRFSGSGSGTDFTLTINSLEAEDAAAYYCLQYSSSPWTFGPGTKVDIKRTVAAPSVFIFPPSDEQLKSGTASVVCLLNNFYPREAKVQWKVDNALQSGNSQESVTEQDSKDSTYSLSSTLTLSKADYEKHKVYACEVTHQGLSSPVTKSFNRGEC

SEQ ID NO: 10 - protein, 214 aa, synthetic construct
  source 1..214: note = Immunoglobulin IgG light chain to the insulin receptor LFR3
DIQLTQSPSSLSASVGDRVTITCRASQDIGGNLYWYQQKPGKAPKVLIYATSSLDSGVPSRFSGSGSGTDFTLTISSLQPEDFATYYCLQYSSSPWTFGQGTKVEIKRTVAAPSVFIFPPSDEQLKSGTASVVCLLNNFYPREAKVQWKVDNALQSGNSQESVTEQDSKDSTYSLSSTLTLSKADYEKHKVYACEVTHQGLSSPVTKSFNRGEC

SEQ ID NO: 11 - protein, 214 aa, synthetic construct
  source 1..214: note = Immunoglobulin IgG light chain to the insulin receptor LFR4
EIVLTQSPATLSLSPGERATLSCRASQDIGGNLYWYQQKPGQAPRLLIYATSSLDSGIPARFSGSGSGTDFTLTISSLEPEDFAVYYCLQYSSSPWTFGQGTRLEIKRTVAAPSVFIFPPSDEQLKSGTASVVCLLNNFYPREAKVQWKVDNALQSGNSQESVTEQDSKDSTYSLSSTLTLSKADYEKHKVYACEVTHQGLSSPVTKSFNRGEC

SEQ ID NO: 12 - protein, 748 aa, synthetic construct
  source 1..748: note = Fragment VH-CH1 of the immunoglobulin heavy chain to the human insulin receptor coupled to the iduronate-2-sulfatase sequence HFR1
EVQLVESGGGLVQPGRSLRLSCAASGFTFTNYDIHWVRQAPGKGLEWVSWIYPGDGSTKYNEKFKGRFTISRDNAKNSLYLQMNSLRAEDTAVYYCAKEWAYWGQGTLVTVSSASTKGPSVFPLAPSSKSTSGGTAALGCLVKDYFPEPVTVSWNSGALTSGVHTFPAVLQSSGLYSLSSVVTVPSSSLGTQTYICNVNHKPSNTKVDKKVEPKSCDKTHLSSSETQANSTTDALNVLLIIVDDLRPSLGCYGDKLVRSPNIDQLASHSLLFQNAFAQQAVCAPSRVSFLTGRRPDTTRLYDFNSYWRVHAGNFSTIPQYFKENGYVTMSVGKVFHPGISSNHTDDSPYSWSFPPYHPSSEKYENTKTCRGPDGELHANLLCPVDVLDVPEGTLPDKQSTEQAIQLLEKMKTSASPFFLAVGYHKPHIPFRYPKEFQKLYPLENITLAPDPEVPDGLPPVAYNPWMDIRQREDVQALNISVPYGPIPVDFQRKIRQSYFASVSYLDTQVGRLLSALDDLQLANSTIIAFTSDHGWALGEHGEWAKYSNFDVATHVPLIFYVPGRTASLPEAGEKLFPYLDPFDSASQLMEPGRQSMDLVELVSLFPTLAGLAGLQVPPRCPVPSFHVELCREGKNLLKHFRFRDLEEDPYLPGNPRELIAYSQYPRPSDIPQWNSDKPSLKDIKIMGYSIRTIDYRYTVWVGFNPDEFLANFSDIHAGELYFVDSDPLQDHNMYNDSQGGDLFQLLMP

SEQ ID NO: 13 - protein, 748 aa, synthetic construct
  source 1..748: note = Fragment VH-CH1 of the immunoglobulin heavy chain to the human insulin receptor coupled to the iduronate-2-sulfatase sequence HFR2
QVQLVESGGGVVQPGRSLRLSCAASGFTFSNYDIHWVRQAPGKGLEWVAWIYPGDGSTKYNEKFKGRFTISRDNSKNTLYLQMNGLRAEDTAVYYCAREWAYWGQGTLVTVSSASTKGPSVFPLAPSSKSTSGGTAALGCLVKDYFPEPVTVSWNSGALTSGVHTFPAVLQSSGLYSLSSVVTVPSSSLGTQTYICNVNHKPSNTKVDKRVEPKSCDKTHLSSSETQANSTTDALNVLLIIVDDLRPSLGCYGDKLVRSPNIDQLASHSLLFQNAFAQQAVCAPSRVSFLTGRRPDTTRLYDFNSYWRVHAGNFSTIPQYFKENGYVTMSVGKVFHPGISSNHTDDSPYSWSFPPYHPSSEKYENTKTCRGPDGELHANLLCPVDVLDVPEGTLPDKQSTEQAIQLLEKMKTSASPFFLAVGYHKPHIPFRYPKEFQKLYPLENITLAPDPEVPDGLPPVAYNPWMDIRQREDVQALNISVPYGPIPVDFQRKIRQSYFASVSYLDTQVGRLLSALDDLQLANSTIIAFTSDHGWALGEHGEWAKYSNFDVATHVPLIFYVPGRTASLPEAGEKLFPYLDPFDSASQLMEPGRQSMDLVELVSLFPTLAGLAGLQVPPRCPVPSFHVELCREGKNLLKHFRFRDLEEDPYLPGNPRELIAYSQYPRPSDIPQWNSDKPSLKDIKIMGYSIRTIDYRYTVWVGFNPDEFLANFSDIHAGELYFVDSDPLQDHNMYNDSQGGDLFQLLMP

SEQ ID NO: 14 - protein, 748 aa, synthetic construct
  source 1..748: note = Fragment VH-CH1 of the immunoglobulin heavy chain to the human insulin receptor coupled to the iduronate-2-sulfatase sequence HFR3
EVQLVESGGGLVQPGGSLRLSCAASGYDFTNYDIHWVRQAPGKGLEWVGWIYPGDGSTKYNEKFKGRFTFSLDTSKSTAYLQMNSLRAEDTAVYYCAKEWAYWGQGTLVTVSSASTKGPSVFPLAPSSKSTSGGTAALGCLVKDYFPEPVTVSWNSGALTSGVHTFPAVLQSSGLYSLSSVVTVPSSSLGTQTYICNVNHKPSNTKVDKKVEPKSCDKTHLSSSETQANSTTDALNVLLIIVDDLRPSLGCYGDKLVRSPNIDQLASHSLLFQNAFAQQAVCAPSRVSFLTGRRPDTTRLYDFNSYWRVHAGNFSTIPQYFKENGYVTMSVGKVFHPGISSNHTDDSPYSWSFPPYHPSSEKYENTKTCRGPDGELHANLLCPVDVLDVPEGTLPDKQSTEQAIQLLEKMKTSASPFFLAVGYHKPHIPFRYPKEFQKLYPLENITLAPDPEVPDGLPPVAYNPWMDIRQREDVQALNISVPYGPIPVDFQRKIRQSYFASVSYLDTQVGRLLSALDDLQLANSTIIAFTSDHGWALGEHGEWAKYSNFDVATHVPLIFYVPGRTASLPEAGEKLFPYLDPFDSASQLMEPGRQSMDLVELVSLFPTLAGLAGLQVPPRCPVPSFHVELCREGKNLLKHFRFRDLEEDPYLPGNPRELIAYSQYPRPSDIPQWNSDKPSLKDIKIMGYSIRTIDYRYTVWVGFNPDEFLANFSDIHAGELYFVDSDPLQDHNMYNDSQGGDLFQLLMP

SEQ ID NO: 15 - protein, 748 aa, synthetic construct
  source 1..748: note = Fragment VH-CH1 of the immunoglobulin heavy chain to the human insulin receptor coupled to the iduronate-2-sulfatase sequence HFR4
EVQLVESGGGLVQPGRSLRLSCAASGFTFNNYDIHWVRQAPGKGLEWVSWIYPGDGSTKYNEKFKGRFTISRDNAKKSLYLQMNSLRAEDTALYYCAKEWAYWGQGTTVTVSSASTKGPSVFPLAPGSSKSTSGTAALGCLVKDYFPEPVTVSWNSGALTSGVHTFPAVLQSSGLYSLSSVVTVPSSSLGTQTYICNVNHKPSNTKVDKKVEPKSCDKTHLSSSETQANSTTDALNVLLIIVDDLRPSLGCYGDKLVRSPNIDQLASHSLLFQNAFAQQAVCAPSRVSFLTGRRPDTTRLYDFNSYWRVHAGNFSTIPQYFKENGYVTMSVGKVFHPGISSNHTDDSPYSWSFPPYHPSSEKYENTKTCRGPDGELHANLLCPVDVLDVPEGTLPDKQSTEQAIQLLEKMKTSASPFFLAVGYHKPHIPFRYPKEFQKLYPLENITLAPDPEVPDGLPPVAYNPWMDIRQREDVQALNISVPYGPIPVDFQRKIRQSYFASVSYLDTQVGRLLSALDDLQLANSTIIAFTSDHGWALGEHGEWAKYSNFDVATHVPLIFYVPGRTASLPEAGEKLFPYLDPFDSASQLMEPGRQSMDLVELVSLFPTLAGLAGLQVPPRCPVPSFHVELCREGKNLLKHFRFRDLEEDPYLPGNPRELIAYSQYPRPSDIPQWNSDKPSLKDIKIMGYSIRTIDYRYTVWVGFNPDEFLANFSDIHAGELYFVDSDPLQDHNMYNDSQGGDLFQLLMP